European Patent Specification EP 4 045 911 B1, published January 28, 2026. Title: Microbiome-Based Informed Method to Formulate Live Biotherapeutics. Applicant: Ravel, Jacques France, Michael Rutt, Lindsay Ma, Bing. Application Not yet assigned. The sequence listing filed with the application follows.

SEQUENCE LISTING (6 sequences)

SEQ ID NO: 1 - DNA, 1950 bp, Lactobacillus crispatus
atgtgcggaattgtcgcattttatgatccaaaaataaacgaaaaacaagccgttattggtaagatgatggctactatcaagcaccgtggacctaattccgacggttattacactaatgatgaggttgcccttggtttcagaagattgtcaattatcgatcttcgtgggggagctcaacctatttataatgaagataaaactagagcaattatctttaatggtgaaatttacaactttaaaccattaagagaacaattaattaaagcaggccacactttcactaccaaggccgatactgaagtattgcttcacggttatgaagagtggggcatggatggccttcttaagaaggtacgtggtatgtttgccttccttatttgggatgacaacaacaagaccctttatggtgcacgtgacttctttggtattaagccaatgtactacagcaaccaagatggccacttacttgtaggttcagaacttaagagtttcttggaatatccaaagttcaagcgtgaattgaacgttgaagctgttaagccatacctcatgaaccaatacaacgaccttgaagaaaccttctttaaaggcgtttacagattcccagcaggtcactggttcgaatacaaagatggtgaaatgaagacccaccaatactgggatgcggaatacaaggaaaatagtttaagctttgaagaaactttgaagcgtatcaacgatgacttgaaggaaaccgttgatttgtacagaattgctgacgttaaggttggtgcattcttgtcagaaggtattgactcttcatacttgactactttgcttaacccagacgatgttttctcagtaagttttgatgactcaacttacgatgaagcttcaaaggctaaggcattagctgacatcaaccactggaagttctacagtgacaaggttgatgccgacgaagctatgcgtgattttccagaaatgcaataccacatggatgaaccagatgccaacccatcaatcatcccactttggtacttgtgtaagttagctcgtaagcacgttactgttgcactttctggtgaaggtgccgacgaattatttgctggctacgttaactacgggatgcatacgcataacgacattattaaggtctttacttcagaattgaaaaagttgcctgagaagaagcgggttaaattggcacacaagattaagagaatgcctaatttcccaggtaaagttcacatgtacaccaatttagctgaaccgagtgaattttatgtcggtcaatcggttatctatgacatggattacccaactatctttacttctaaagatgctaatagcattttacagccaacgtatcgcaataaattgactgttaacggcatttaccaaaaagactttaagaaagtaaagggagtcgataatgttaagcagatgcaatacattgacttgcaccactttatgcttaacgatattgaacaaaaagctgataagatttcgatggcccattcacttgaagttcgtgttccttacctcgacaagaagattgcggaattggctaactctatcccaaccaagtacttggttaaccgtcatgataccaagtatgctttgcgtaaggcttcagaaaaagttttaccagatgagtgggctaagagacctaagcttggcttcccaactccaattaagcaatggttgaaggaaccacgtttttacaaacaagttcatgctctttttgaagaagaatttgtcaacgatatttttgaccaaaagaagattatcaagttacttgacgacaactatgaaggtgatggctcacatagacgtcaaatctgggctatctacaccttccttgtttggtacaagttgttctttgttgattacgaaaacacagttaagaaatatcaacacgtgcaacctgaagttgctaagctaatttcacagggcaaattactataa

SEQ ID NO: 2 - DNA, 1950 bp, Lactobacillus crispatus
atgtgcggaattgtcgcgttttatgatccaaagataaatgaaaagcaggctgtcattggcaaaatgatggccacgattaaacaccgcggacctagttccgacgggtattatactaatgacgaggttgcccttggttttagaagattatcaattattgatcttcgtgggggtagccaacctatttataatgaagataaaactagagcaattatttttaatggtgaaatttataactttaagccattaagagaagaattaattaaagcaggccatgattttactactaaggctgatacagaagtcttacttcatggttatgaagaatggggcatggatggcttgcttaagcgtgtacgtgggatgttcgccttcttaatttgggatgacaacaacaagaccctttatggtgcacgtgacttctttggcattaagccaatgtactacagtaatcaaaatggccatttgttggttggttcagaattaaagagctttttggaatttccaaagttcaagcgggaattaaatgttgaagcagttaagccatacttgatgaatcaatacaatgacctagaagaaaccttctttaagggcgtttaccgcttcccagcgggccattggtttgaatacaaagatggtgaaatgaagacccatcaatattgggatgctgaatataaagaaaatagcctttcctttgaagaaactttgcaaaagatcaacgaagatttgaaagaaacggttgatttgtatagaaacgctgatgttaaggttggtgctttcttatcagaaggaatcgactcttcatacttgactagtttgcttaacccagatgacgttttctcagtaagttttgatgattcaacttatgatgaagcttctaaggctaaggcattagcagatattaatcactggaagttcttcagcgataaggttgatgctgatgaagcaatgcgtgacttcccagaaatgcaataccacatggatgaaccagatgctaatccgtcaatcattccactctggtacttgtgtaaactagctcgtaagcatgttactgttgctctttcaggtgaaggcgctgatgaattgtttgctggttatgtgaactacgggatgcatacgcataacgacattattaaggtctttacttcagaattgaaaaagttgcctgagaagaagcgggttaaattggcacacaagattaagagaatgcctaatttcccaggtaaagttcacatgtacaccaatttagctgaaccgagtgaattttatgtcggtcaatcggttatctatgacatggattacccaactatctttacttctaaagatgctaatagcattttacagccaacgtatcgcaataaattgactgttaacggcatttaccaaaaagactttaagaaagtaaagggagtcgataatgttaagcagatgcaatacattgacttgcaccactttatgcttaacgatattgaacaaaaagctgataagatttcgatggcccattcacttgaagttcgtgttccttacctcgacaagaagattgcggaattggctaactctatcccaaccaagtacttggttaaccgtcatgataccaagtatgctttgcgtaaggcttcagaaaaagttttaccagatgagtgggctaagagacctaagcttggcttcccaactccaattaagcaatggttgaaggaaccacgtttttacaaacaagttcatgctctttttgaagaagaatttgtcaacgatatttttgaccaaaagaagattatcaagttacttgacgacaactatgaaggtgatggctcacatagacgtcaaatctgggctatctataccttccttgtttggtacaagttgttctttgttgattacgaaaacacagttaagaaatatcaacacgtgcaacctgaagttgctaagctaatttcacagggtaaattactataa

SEQ ID NO: 3 - DNA, 1948 bp, Lactobacillus crispatus
atgtgcggaattgtcgcgttttatgatccaaagataaatgaaaagcaggctgtcattggcaaaatgatggccacgattaaacaccgcggacctagttccgacgggtattatactaatgacgaggttgcccttggttttagaagattatcaattattgatcttcgtgggggtagccaacctatttataatgaagataaaactagagcaattatttttaatggtgaaatttataactttaagccattaagagaagaattaattaaagcaggccatgattttactactaaggctgatacagaagtcttacttcatggttatgaagaatggggcatggatggcttgcttaagcgtgtacgtgggatgttcgccttcttaatttgggatgacaacaacaagaccctttatggtgcacgtgacttctttggcattaagccaatgtactacagtaatcaaaatggccatttgttggttggttcagaattaaagagctttttggaatttccaaagttcaagcgggaattaaatgttgaagcagttaagccatacttgatgaatcaatacaatgacctagaagaaaccttctttaagggcatttaccgcttcccagcgggccattggtttgaatacaaagatggtgaaatgaagacccatcaatattgggatgctgaatataaagaaaatagcctttcctttgaagaaactttgcaaaagatcaacgaagatttgaaagaaacggttgatttgtatagaaacgctgatgttaaggttggtgctttcttatcagaaggaatcgactcttcatacttgactagtttgcttaacccagatgacgttttctcagtaagttttgatgattcaacttatgatgaagcttctaaggctaaggcattagcagatattaatcctggaagttcttcagcgatmggttgatgctgatgaagcaatgcgtgacttcccagaaatgcaataccacatggatgaaccagatgctaatccgtcaatcattccactctggtacttgtgtaaactagctcgtaagcatgttactgttgctctttcaggtgaaggcgctgatgaattgtttgctggttatgtgaactacgggatgcatacgcataacgacattattaaggtctttacttcagaattgaaaaagttgcctgagaagaagcgggttaaattggcacacaagattaagagaatgcctaatttcccaggtaaagttcacatgtacaccaatttagctgaaccgagtgaattttatgtcggtcaatcggttatctatgacatggattacccaactatctttacttctaaagatgctaatagcattttacagccaacgtatcgcaataaattgactgttaacggcatttaccaaaaagactttaagaaagtaaagggagtcgataatgttaagcagatgcaatacattgacttgcaccactttatgcttaacgatattgaacaaaaagctgataagatttcgatggcccattcacttgaagttcgtgttccttacctcgacaagaagattgcggaattggctaactctatcccaaccaagtacttggttaaccgtcatgataccaagtatgctttgcgtaaggcttcagaaaaagttttaccagatgagtgggctaagagacctaagcttggcttcccaactccaattaagcaatggttgaaggaaccacgtttttacaaacaagttcatgctctttttgaagaagaatttgtcaacgatatttttgaccaaaagaagattatcaagttacttgacgacaactatgaaggtgatggctcacatagacgtcaaatctgggctatctataccttccttgtttggtacaagttgttctttgttgattacgaaaacacagttaagaaatatcaacacgtgcaacctgaagttgctaagctaatttcacagggtaaattactataa

SEQ ID NO: 4 - protein, 650 aa, Lactobacillus crispatus
MCGIVAFYDPKINEKQAVIGKMMATIKHRGPNSDGYYTNDEVALGFRRLSIIDLRGGAQPIYNEDKTRAIIFNGEIYNFKPLREQLIKAGHTFTTKADTEVLLHGYEEWGMDGLLKKVRGMFAFLIWDDNNKTLYGARDFFGIKPMYYSNQDGHLLVGSELKSFLEYPKFKRELNVEAVKPYLMNQYNDLEETFFKGWRFPAGHWFEYKDGEMKTHQYWDAEYKENSLSFEETLKRINDDLKETVDLYRIADVKVGAFLSEGIDSSYLTTLLNPDDVFSVSFDDSTYDEASKAKALADINHLALKFYSDKVDADEAMRDFPEMQYHMDEPDANPSIIPLWYLCKLARKHVTVALSGEGADELFAGYVNYGMHTHNDIIKVFTSELKKLPEKKRVKLAHKIKRMPNFPGKVHMYTNLAEPSEFYVGQSVIYDMDYPTIFTSKDANSILQPTYRNKLTVNGIYQKDFKKVKGVDNVKQMQYIDLHHFMLNDIEQKADKISMAHSLEVRVPYLDKKIAELANSIPTKYLVNRHDTKYALRKASEKVLPDEWAKRPKLGFPTPIKQWLKEPRFYKQVHALFEEEFVNDIFDQKKIIKLLDDNYEGDGSHRRQIWAIYTFLVWYKLFFVDYENTVKKYQHVQPEVAKLISQGKLL

SEQ ID NO: 5 - protein, 651 aa, Lactobacillus crispatus
MCGIVAFYDPKINEKQAVIGKMMATIKHRGPSSDGYYTNDEVALGFRRLSIIDLRGGSQPIYNEDKTRAIIFNGEIYNFKPLREELIKAGHDFTTKADTEVLLHGYEEWGMDGLLKRVRGMFAFLIWDDNNKTLYGARDFFGIKPMYYSNQNGHLLVGSELKSFLEFPKFKRELNVEAVKPYLMNQYNDLEETFFKGVYRFPAGHWFEYKDGEMKTHQYLALDAEYKENSLSFEETLQKINEDLKETVDLYRNADVKVGAFLSEGIDSSYLTSLLNPDDVFSVSFDDSTYDEASKAKALADINHWKFFSDKVDADEAMRDFPEMQYHMDEPDANPSIIPLWYLCKLARKHVTVALSGEGADELFAGYVNYGMHTHNDIIKVFTSELKKLPEKKRVKLAHKIKRMPNFPGKVHMYTNLAEPSEFYVGQSVIYDMDYPTIFTSKDANSILQPTYRNKLTVNGIYQKDFKKVKGVDNVKQMQYIDLHHFMLNDIEQKADKISMAHSLEVRVPYLDKKIAELANSIPTKYLVNRHDTKYALRKASEKVLPDEWAKRPKLGFPTPIKQWLKEPRFYKQVHALFEEEFVNDIFDQKKIIKLLDDNYEGDGSHRRQIWAIYTFLVWYKLFFVDYENTVKKYQHVQPEVAKLISQGKLL

SEQ ID NO: 6 - protein, 651 aa, Lactobacillus crispatus
MCGIVAFYDPKINEKQAVIGKMMATIKHRGPSSDGYYTNDEVALGFRRLSIIDLRGGSQPIYNEDKTRAIIFNGEIYNFKPLREELIKAGHDFTTKADTEVLLHGYEEWGMDGLLKRVRGMFAFLIWDDNNKTLYGARDFFGIKPMYYSNQNGHLLVGSELKSFLEFPKFKRELNVEAVKPYLMNQYNDLEETFFKGIYRFPAGHWFEYKDGEMKTHQYWDAEYKENSLSFEETLQKINEDLKETVDLYRNADVKVGAFLSEGIDSSYLTSLLNPDDVFSVSFDDSTYDEASKAKALADINHWKFFSDKVDADEAMRDFPEMQYHMDEPDANPSIIPLWYLCKLARKHVTVALSGEGADELFAGYVNYGMHTHNDIIKVFTSELKKLPEKKRVKLAHKIKRMPNFPGKVHMYTNLAEPSEFYVGQSVIYDMDYPTIFTSKDANSILQPTYRNKLTVNGIYQKDFKKVKGVDNVKQMQYIDLHHFMLNDIEQKADKISMAHSLEVRVPYLDKKIAELANSIPTKYLVNRHDTKYALRKASEKVLPDEWAKRPKLGFPTPIKQWLKEPRFYKQVHALFEEEFVNDIFDQKKIIKLLDDNYEGDGSHRRQIWAIYTFLVLALYKLFFVDYENTVKKYQHVQPEVAKLISQGKLL